European Patent Application EP 4 512 426 A1, published February 26, 2025. Title: COMPOUND AND USE THEREOF. Applicant: COHERENT BIOPHARMA (SUZHOU) LIMITED. The sequence listing filed with the application follows.

SEQUENCE LISTING (4 sequences)

SEQ ID NO: 1 - protein, 13 aa, synthetic construct
KEFLHPSKVDLPR

SEQ ID NO: 2 - protein, 27 aa, synthetic construct
EGKLSSNDTEGGLCKEFLHPSKVDLPR

SEQ ID NO: 3 - protein, 17 aa, synthetic construct
  SITE 2: note = X is N, H, or Y
  SITE 4: note = X is G, S, T, or N
  SITE 8: note = X is T or R
  SITE 15: note = X is A, D, E, G, or S
  SITE 16: note = X is S or T
  SITE 17: note = X is D or E
  SITE 1..13: note = disulfide bond
  SITE 3..11: note = disulfide bond
CXCXGPPXFECWCYXXX

SEQ ID NO: 4 - protein, 26 aa, synthetic construct
  SITE 4..16: note = disulfide bond
  SITE 6..14: note = disulfide bond
AGSCYCSGPPRFECWCYETEGTGGGK